European Patent Specification EP 3 442 567 B1, published December 3, 2025. Title: Anti-PSMA antibodies and use thereof. Applicant: Zhao, Aizhi Wen, Weihong Han, Yueheng. The sequence listing filed with the application follows.

SEQUENCE LISTING (116 sequences)

SEQ ID NO: 1 - protein, 707 aa, Homo sapiens
KSSNEATNITPKHNMKAFLDELKAENIKKFLYNFTQIPHLAGTEQNFQLAKQIQSQWKEFGLDSVELAHYDVLLSYPNKTHPNYISIINEDGNEIFNTSLFEPPPPGYENVSDIVPPFSAFSPQGMPEGDLVYVNYARTEDFFKLERDMKINCSGKIVIARYGKVFRGNKVKNAQLAGAKGVILYSDPADYFAPGVKSYPDGWNLPGGGVQRGNILNLNGAGDPLTPGYPANEYAYRRGIAEAVGLPSIPVHPIGYYDAQKLLEKMGGSAPPDSSWRGSLKVPYNVGPGFTGNFSTQKVKMHIHSTNEVTRIYNVIGTLRGAVEPDRYVILGGHRDSWVFGGIDPQSGAAVVHEIVRSFGTLKKEGWRPRRTILFASWDAEEFGLLGSTEWAEENSRLLQERGVAYINADSSIEGNYTLRVDCTPLMYSLVHNLTKELKSPDEGFEGKSLYESWTKKSPSPEFSGMPRISKLGSGNDFEVFFQRLGIASGRARYTKNWETNKFSGYPLYHSVYETYELVEKFYDPMFKYHLTVAQVRGGMVFELANSIVLPFDCRDYAVVLRKYADKIYSISMKHPQEMKTYSVSFDSLFSAVKNFTEIASKFSERLQDFDKSNPIVLRMMNDQLMFLERAFIDPLGLPDRPFYRHVIYAPSSHNKYAGESFPGIYDALFDIESKVDPSKAWGEVKRQIYVAAFTVQAAAETLSEVA

SEQ ID NO: 2 - DNA, 756 bp, Artificial Sequence
  scFv
cagtctgtgctgactcagccgccctcagtgtctggggccccagggcagagtgtcattatctcctgcactgggagcagctccaacatcggggcaggttctcatgtacactggtaccagcaggttccaggaacagcccccaaactcctcatctatggaaacaccaatcggccctcaggggtccctgaccgattctctggctccaagtctggcacctcaggttccctggccatcactggactccagcctgaggatgaggctgattattattgtgcaacatgggatgacagtctgaatggtgtaatattcggcggagggaccaaggtcaccgtcctaggcggatcctctaggtcaagttccagcggcggcggtggcagcggaggcggcggtgaggtgcagctggtggagtctgggggagccctggccaagcctggggggtccctgagactctcctgtgcagcctctggatccaccctcagtggctatgctatgcactgggtccgccaggctccaggcaaggggctggagtgggtggcagttatatcatatgatggaagcaataaatactacgcagactccgtgaagggccgattcaccatctccagagacaattccaagaacacgctgtttctgcaaatgaacagcctgagacctgaggacacggctgtgtactattgtgctaaaggccttacttggggactcggtgacaatgatgctctcgatatctggggccccgggaccacggtcaccgtctcctca

SEQ ID NO: 3 - protein, 252 aa, Artificial Sequence
  scFv
QSVLTQPPSVSGAPGQSVIISCTGSSSNIGAGSHVHWYQQVPGTAPKLLIYGNTNRPSGVPDRFSGSKSGTSGSLAITGLQPEDEADYYCATWDDSLNGVIFGGGTKVTVLGGSSRSSSSGGGGSGGGGEVQLVESGGALAKPGGSLRLSCAASGSTLSGYAMHWVRQAPGKGLEWVAVISYDGSNKYYADSVKGRFTISRDNSKNTLFLQMNSLRPEDTAVYYCAKGLTWGLGDNDALDIWGPGTTVTVSS

SEQ ID NO: 4 - DNA, 333 bp, Homo sapiens
cagtctgtgctgactcagccgccctcagtgtctggggccccagggcagagtgtcattatctcctgcactgggagcagctccaacatcggggcaggttctcatgtacactggtaccagcaggttccaggaacagcccccaaactcctcatctatggaaacaccaatcggccctcaggggtccctgaccgattctctggctccaagtctggcacctcaggttccctggccatcactggactccagcctgaggatgaggctgattattattgtgcaacatgggatgacagtctgaatggtgtaatattcggcggagggaccaaggtcaccgtccta

SEQ ID NO: 5 - protein, 111 aa, Homo sapiens
QSVLTQPPSVSGAPGQSVIISCTGSSSNIGAGSHVHWYQQVPGTAPKLLIYGNTNRPSGVPDRFSGSKSGTSGSLAITGLQPEDEADYYCATWDDSLNGVIFGGGTKVTVL

SEQ ID NO: 6 - DNA, 75 bp, Homo sapiens
cagtctgtgctgactcagccgccctcagtgtctggggccccagggcagagtgtcattatctcctgcactgggagc

SEQ ID NO: 7 - protein, 25 aa, Homo sapiens
QSVLTQPPSVSGAPGQSVIISCTGS

SEQ ID NO: 8 - DNA, 27 bp, Homo sapiens
agctccaacatcggggcaggttctcat

SEQ ID NO: 9 - protein, 9 aa, Homo sapiens
SSNIGAGSH

SEQ ID NO: 10 - DNA, 51 bp, Homo sapiens
gtacactggtaccagcaggttccaggaacagcccccaaactcctcatctat

SEQ ID NO: 11 - protein, 17 aa, Homo sapiens
VHWYQQVPGTAPKLLIY

SEQ ID NO: 12 - DNA, 9 bp, Homo sapiens
ggaaacacc

SEQ ID NO: 13 - protein, 3 aa, Homo sapiens
GNT

SEQ ID NO: 14 - DNA, 108 bp, Homo sapiens
aatcggccctcaggggtccctgaccgattctctggctccaagtctggcacctcaggttccctggccatcactggactccagcctgaggatgaggctgattattattgt

SEQ ID NO: 15 - protein, 36 aa, Homo sapiens
NRPSGVPDRFSGSKSGTSGSLAITGLQPEDEADYYC

SEQ ID NO: 16 - DNA, 33 bp, Homo sapiens
gcaacatgggatgacagtctgaatggtgtaata

SEQ ID NO: 17 - protein, 11 aa, Homo sapiens
ATWDDSLNGVI

SEQ ID NO: 18 - DNA, 30 bp, Homo sapiens
ttcggcggagggaccaaggtcaccgtccta

SEQ ID NO: 19 - protein, 10 aa, Homo sapiens
FGGGTKVTVL

SEQ ID NO: 20 - DNA, 369 bp, Homo sapiens
gaggtgcagctggtggagtctgggggagccctggccaagcctggggggtccctgagactctcctgtgcagcctctggatccaccctcagtggctatgctatgcactgggtccgccaggctccaggcaaggggctggagtgggtggcagttatatcatatgatggaagcaataaatactacgcagactccgtgaagggccgattcaccatctccagagacaattccaagaacacgctgtttctgcaaatgaacagcctgagacctgaggacacggctgtgtactattgtgctaaaggccttacttggggactcggtgacaatgatgctctcgatatctggggccccgggaccacggtcaccgtctcctca

SEQ ID NO: 21 - protein, 123 aa, Homo sapiens
EVQLVESGGALAKPGGSLRLSCAASGSTLSGYAMHWVRQAPGKGLEWVAVISYDGSNKYYADSVKGRFTISRDNSKNTLFLQMNSLRPEDTAVYYCAKGLTWGLGDNDALDIWGPGTTVTVSS

SEQ ID NO: 22 - DNA, 75 bp, Homo sapiens
gaggtgcagctggtggagtctgggggagccctggccaagcctggggggtccctgagactctcctgtgcagcctct

SEQ ID NO: 23 - protein, 25 aa, Homo sapiens
EVQLVESGGALAKPGGSLRLSCAAS

SEQ ID NO: 24 - DNA, 24 bp, Homo sapiens
ggatccaccctcagtggctatgct

SEQ ID NO: 25 - protein, 8 aa, Homo sapiens
GSTLSGYA

SEQ ID NO: 26 - DNA, 51 bp, Homo sapiens
atgcactgggtccgccaggctccaggcaaggggctggagtgggtggcagtt

SEQ ID NO: 27 - protein, 17 aa, Homo sapiens
MHWVRQAPGKGLEWVAV

SEQ ID NO: 28 - DNA, 24 bp, Homo sapiens
atatcatatgatggaagcaataaa

SEQ ID NO: 29 - protein, 8 aa, Homo sapiens
ISYDGSNK

SEQ ID NO: 30 - DNA, 114 bp, Homo sapiens
tactacgcagactccgtgaagggccgattcaccatctccagagacaattccaagaacacgctgtttctgcaaatgaacagcctgagacctgaggacacggctgtgtactattgt

SEQ ID NO: 31 - protein, 38 aa, Homo sapiens
YYADSVKGRFTISRDNSKNTLFLQMNSLRPEDTAVYYC

SEQ ID NO: 32 - DNA, 48 bp, Homo sapiens
gctaaaggccttacttggggactcggtgacaatgatgctctcgatatc

SEQ ID NO: 33 - protein, 16 aa, Homo sapiens
AKGLTWGLGDNDALDI

SEQ ID NO: 34 - DNA, 33 bp, Homo sapiens
tggggccccgggaccacggtcaccgtctcctca

SEQ ID NO: 35 - protein, 11 aa, Homo sapiens
WGPGTTVTVSS

SEQ ID NO: 36 - DNA, 54 bp, Artificial Sequence
  linker
ggcggatcctctaggtcaagttccagcggcggcggtggcagcggaggcggcggt

SEQ ID NO: 37 - protein, 18 aa, Artificial Sequence
  linker
GGSSRSSSSGGGGSGGGG

SEQ ID NO: 38 - DNA, 51 bp, Artificial Sequence
  mutant
gtacactggtaccagcaggctccaggaacagcccccaaactcctcatctat

SEQ ID NO: 39 - protein, 17 aa, Artificial Sequence
  mutant
VHWYQQAPGTAPKLLIY

SEQ ID NO: 40 - DNA, 9 bp, Artificial Sequence
  mutant
gaaaacacc

SEQ ID NO: 41 - protein, 3 aa, Artificial Sequence
  mutant
ENT

SEQ ID NO: 42 - DNA, 30 bp, Artificial Sequence
  mutant
ttcggcggagggaccaaggccaccgtccta

SEQ ID NO: 43 - protein, 10 aa, Artificial Sequence
  mutant
FGGGTKATVL

SEQ ID NO: 44 - DNA, 24 bp, Artificial Sequence
  mutant
ggattcaccctcagtggctatgct

SEQ ID NO: 45 - protein, 8 aa, Artificial Sequence
  mutant
GFTLSGYA

SEQ ID NO: 46 - DNA, 114 bp, Artificial Sequence
  mutant
tactacgcagactccgtgaagggccgattcaccgtctccagagacaattccaagaacacgctgtttctgcaaatgaacagcctgagacctgaggacacggctgtgtactattgt

SEQ ID NO: 47 - protein, 38 aa, Artificial Sequence
  mutant
YYADSVKGRFTVSRDNSKNTLFLQMNSLRPEDTAVYYC

SEQ ID NO: 48 - DNA, 48 bp, Artificial Sequence
  mutant
gctaaaggccttacttggggactcggtgacaatgatgctctcggtatc

SEQ ID NO: 49 - protein, 16 aa, Artificial Sequence
  mutant
AKGLTWGLGDNDALGI

SEQ ID NO: 50 - DNA, 33 bp, Artificial Sequence
  mutant
tggggccccgagaccacggtcaccgtctcctca

SEQ ID NO: 51 - protein, 11 aa, Artificial Sequence
  mutant
WGPETTVTVSS

SEQ ID NO: 52 - DNA, 1419 bp, Homo sapiens
atggagtttgggctgagctgggttttcctcgttgctcttttaagaggtgtccagtgtgaggtgcagctggtggagtctgggggagccctggccaagcctggggggtccctgagactctcctgtgcagcctctggattcaccctcagtggctatgctatgcactgggtccgccaggctccaggcaaggggctggagtgggtggcagttatatcatatgatggaagcaataaatactacgcagactccgtgaagggccgattcaccgtctccagagacaattccaagaacacgctgtttctgcaaatgaacagcctgagacctgaggacacggctgtgtactattgtgctaaaggccttacctggggactcggtgacaatgatgctctcgatatctggggccccgggaccacggtcaccgtctcctcagcctccaccaagggcccatcggtcttccccctggcaccctcctccaagagcacctctgggggcacagcggccctgggctgcctggtcaaggactacttccccgaaccggtgacggtgtcgtggaactcaggcgccctgaccagcggcgtgcacaccttcccggctgtcctacagtcctcaggactctactccctcagcagcgtggtgaccgtgccctccagcagcttgggcacccagacctacatctgcaacgtgaatcacaagcccagcaacaccaaggtggacaagaaagttgagcccaaatcttgtgacaaaactcacacatgcccaccgtgcccagcacctgaactcctggggggaccgtcagtcttcctcttccccccaaaacccaaggacaccctcatgatctcccggacccctgaggtcacatgcgtggtggtggacgtgagccacgaagaccctgaggtcaagttcaactggtacgtggacggcgtggaggtgcataatgccaagacaaagccgcgggaggagcagtacaacagcacgtaccgggtggtcagcgtcctcaccgtcctgcaccaggactggctgaatggcaaggagtacaagtgcaaggtctccaacaaagccctcccagcccccatcgagaaaaccatctccaaagccaaagggcagccccgagaaccacaggtgtacaccctgcccccatcccgggatgagctgaccaagaaccaggtcagcctgacctgcctggtcaaaggcttctatcccagcgacatcgccgtggagtgggagagcaatgggcagccggagaacaactacaagaccacgcctcccgtgctggactccgacggctccttcttcctctacagcaagctcaccgtggacaagagcaggtggcagcaggggaacgtcttctcatgctccgtgatgcatgaggctctgcacaaccactacacgcagaagagcctctccctgtctccgggtaaatga

SEQ ID NO: 53 - protein, 472 aa, Homo sapiens
MEFGLSWVFLVALLRGVQCEVQLVESGGALAKPGGSLRLSCAASGFTLSGYAMHWVRQAPGKGLEWVAVISYDGSNKYYADSVKGRFTVSRDNSKNTLFLQMNSLRPEDTAVYYCAKGLTWGLGDNDALDIWGPGTTVTVSSASTKGPSVFPLAPSSKSTSGGTAALGCLVKDYFPEPVTVSWNSGALTSGVHTFPAVLQSSGLYSLSSVVTVPSSSLGTQTYICNVNHKPSNTKVDKKVEPKSCDKTHTCPPCPAPELLGGPSVFLFPPKPKDTLMISRTPEVTCVVVDVSHEDPEVKFNWYVDGVEVHNAKTKPREEQYNSTYRVVSVLTVLHQDWLNGKEYKCKVSNKALPAPIEKTISKAKGQPREPQVYTLPPSRDELTKNQVSLTCLVKGFYPSDIAVEWESNGQPENNYKTTPPVLDSDGSFFLYSKLTVDKSRWQQGNVFSCSVMHEALHNHYTQKSLSLSPGK

SEQ ID NO: 54 - DNA, 57 bp, Homo sapiens
atggagtttgggctgagctgggttttcctcgttgctcttttaagaggtgtccagtgt

SEQ ID NO: 55 - protein, 19 aa, Homo sapiens
MEFGLSWVFLVALLRGVQC

SEQ ID NO: 56 - DNA, 369 bp, Homo sapiens
gaggtgcagctggtggagtctgggggagccctggccaagcctggggggtccctgagactctcctgtgcagcctctggattcaccctcagtggctatgctatgcactgggtccgccaggctccaggcaaggggctggagtgggtggcagttatatcatatgatggaagcaataaatactacgcagactccgtgaagggccgattcaccgtctccagagacaattccaagaacacgctgtttctgcaaatgaacagcctgagacctgaggacacggctgtgtactattgtgctaaaggccttacctggggactcggtgacaatgatgctctcgatatctggggccccgggaccacggtcaccgtctcctca

SEQ ID NO: 57 - protein, 123 aa, Homo sapiens
EVQLVESGGALAKPGGSLRLSCAASGFTLSGYAMHWVRQAPGKGLEWVAVISYDGSNKYYADSVKGRFTVSRDNSKNTLFLQMNSLRPEDTAVYYCAKGLTWGLGDNDALDIWGPGTTVTVSS

SEQ ID NO: 58 - DNA, 990 bp, Homo sapiens
gcctccaccaagggcccatcggtcttccccctggcaccctcctccaagagcacctctgggggcacagcggccctgggctgcctggtcaaggactacttccccgaaccggtgacggtgtcgtggaactcaggcgccctgaccagcggcgtgcacaccttcccggctgtcctacagtcctcaggactctactccctcagcagcgtggtgaccgtgccctccagcagcttgggcacccagacctacatctgcaacgtgaatcacaagcccagcaacaccaaggtggacaagaaagttgagcccaaatcttgtgacaaaactcacacatgcccaccgtgcccagcacctgaactcctggggggaccgtcagtcttcctcttccccccaaaacccaaggacaccctcatgatctcccggacccctgaggtcacatgcgtggtggtggacgtgagccacgaagaccctgaggtcaagttcaactggtacgtggacggcgtggaggtgcataatgccaagacaaagccgcgggaggagcagtacaacagcacgtaccgggtggtcagcgtcctcaccgtcctgcaccaggactggctgaatggcaaggagtacaagtgcaaggtctccaacaaagccctcccagcccccatcgagaaaaccatctccaaagccaaagggcagccccgagaaccacaggtgtacaccctgcccccatcccgggatgagctgaccaagaaccaggtcagcctgacctgcctggtcaaaggcttctatcccagcgacatcgccgtggagtgggagagcaatgggcagccggagaacaactacaagaccacgcctcccgtgctggactccgacggctccttcttcctctacagcaagctcaccgtggacaagagcaggtggcagcaggggaacgtcttctcatgctccgtgatgcatgaggctctgcacaaccactacacgcagaagagcctctccctgtctccgggtaaa

SEQ ID NO: 59 - protein, 330 aa, Homo sapiens [sequence omitted]

SEQ ID NO: 60 - DNA, 711 bp, Homo sapiens
atggcctggtctcctctcctcctcactctcctcgctcactgcacagggtcctgggcccagtctgtgctgactcagccgccctcagtgtctggggccccagggcagagtgtcattatctcctgcactgggagcagctccaacatcggggcaggttctcatgtacactggtaccagcaggttccaggaacagcccccaaactcctcatctatgaaaacaccaatcggccctcaggggtccctgaccgattctctggctccaagtctggcacctcaggttccctggccatcactggactccagcctgaggatgaggctgattattattgtgcaacatgggatgacagtctgaatggtgtaatattcggcggagggaccaaggccaccgtcctaggtcagcccaaggctgccccctcggtcactctgttcccgccctcctctgaggagcttcaagccaacaaggccacactggtgtgtctcataagtgacttctacccgggagccgtgacagtggcctggaaggcagatagcagccccgtcaaggcgggagtggagaccaccacaccctccaaacaaagcaacaacaagtacgcggccagcagctatctgagcctgacgcctgagcagtggaagtcccacagaagctacagctgccaggtcacgcatgaagggagcaccgtggagaagacagtggcccctacagaatgttcatga

SEQ ID NO: 61 - protein, 236 aa, Homo sapiens
MAWSPLLLTLLAHCTGSWAQSVLTQPPSVSGAPGQSVIISCTGSSSNIGAGSHVHWYQQVPGTAPKLLIYENTNRPSGVPDRFSGSKSGTSGSLAITGLQPEDEADYYCATWDDSLNGVIFGGGTKATVLGQPKAAPSVTLFPPSSEELQANKATLVCLISDFYPGAVTVAWKADSSPVKAGVETTTPSKQSNNKYAASSYLSLTPEQWKSHRSYSCQVTHEGSTVEKTVAPTECS

SEQ ID NO: 62 - DNA, 57 bp, Homo sapiens
atggcctggtctcctctcctcctcactctcctcgctcactgcacagggtcctgggcc

SEQ ID NO: 63 - protein, 19 aa, Homo sapiens
MAWSPLLLTLLAHCTGSWA

SEQ ID NO: 64 - DNA, 333 bp, Homo sapiens
cagtctgtgctgactcagccgccctcagtgtctggggccccagggcagagtgtcattatctcctgcactgggagcagctccaacatcggggcaggttctcatgtacactggtaccagcaggttccaggaacagcccccaaactcctcatctatgaaaacaccaatcggccctcaggggtccctgaccgattctctggctccaagtctggcacctcaggttccctggccatcactggactccagcctgaggatgaggctgattattattgtgcaacatgggatgacagtctgaatggtgtaatattcggcggagggaccaaggccaccgtccta

SEQ ID NO: 65 - protein, 111 aa, Homo sapiens
QSVLTQPPSVSGAPGQSVIISCTGSSSNIGAGSHVHWYQQVPGTAPKLLIYENTNRPSGVPDRFSGSKSGTSGSLAITGLQPEDEADYYCATWDDSLNGVIFGGGTKATVL

SEQ ID NO: 66 - DNA, 318 bp, Homo sapiens
ggtcagcccaaggctgccccctcggtcactctgttcccgccctcctctgaggagcttcaagccaacaaggccacactggtgtgtctcataagtgacttctacccgggagccgtgacagtggcctggaaggcagatagcagccccgtcaaggcgggagtggagaccaccacaccctccaaacaaagcaacaacaagtacgcggccagcagctatctgagcctgacgcctgagcagtggaagtcccacagaagctacagctgccaggtcacgcatgaagggagcaccgtggagaagacagtggcccctacagaatgttca

SEQ ID NO: 67 - protein, 106 aa, Homo sapiens
GQPKAAPSVTLFPPSSEELQANKATLVCLISDFYPGAVTVAWKADSSPVKAGVETTTPSKQSNNKYAASSYLSLTPEQWKSHRSYSCQVTHEGSTVEKTVAPTECS

SEQ ID NO: 68 - protein, 453 aa, Homo sapiens
EVQLVESGGALAKPGGSLRLSCAASGFTLSGYAMHWVRQAPGKGLEWVAVISYDGSNKYYADSVKGRFTVSRDNSKNTLFLQMNSLRPEDTAVYYCAKGLTWGLGDNDALDIWGPGTTVTVSSASTKGPSVFPLAPSSKSTSGGTAALGCLVKDYFPEPVTVSWNSGALTSGVHTFPAVLQSSGLYSLSSVVTVPSSSLGTQTYICNVNHKPSNTKVDKKVEPKSCDKTHTCPPCPAPELLGGPSVFLFPPKPKDTLMISRTPEVTCVVVDVSHEDPEVKFNWYVDGVEVHNAKTKPREEQYNSTYRVVSVLTVLHQDWLNGKEYKCKVSNKALPAPIEKTISKAKGQPREPQVYTLPPSRDELTKNQVSLTCLVKGFYPSDIAVEWESNGQPENNYKTTPPVLDSDGSFFLYSKLTVDKSRWQQGNVFSCSVMHEALHNHYTQKSLSLSPGK

SEQ ID NO: 69 - protein, 217 aa, Homo sapiens
QSVLTQPPSVSGAPGQSVIISCTGSSSNIGAGSHVHWYQQVPGTAPKLLIYENTNRPSGVPDRFSGSKSGTSGSLAITGLQPEDEADYYCATWDDSLNGVIFGGGTKATVLGQPKAAPSVTLFPPSSEELQANKATLVCLISDFYPGAVTVAWKADSSPVKAGVETTTPSKQSNNKYAASSYLSLTPEQWKSHRSYSCQVTHEGSTVEKTVAPTECS

SEQ ID NO: 70 - DNA, 63 bp, Homo sapiens
atggccttaccagtgaccgccttgctcctgccgctggccttgctgctccacgccgccaggccg

SEQ ID NO: 71 - protein, 21 aa, Homo sapiens
MALPVTALLLPLALLLHAARP

SEQ ID NO: 72 - DNA, 135 bp, Homo sapiens
accacgacgccagcgccgcgaccaccaacaccggcgcccaccatcgcgtcgcagcccctgtccctgcgcccagaggcgtgccggccagcggcggggggcgcagtgcacacgagggggctggacttcgcctgtgat

SEQ ID NO: 73 - protein, 45 aa, Homo sapiens
TTTPAPRPPTPAPTIASQPLSLRPEACRPAAGGAVHTRGLDFACD

SEQ ID NO: 74 - DNA, 72 bp, Homo sapiens
atctacatctgggcgcccttggccgggacttgtggggtccttctcctgtcactggttatcaccctttactgc

SEQ ID NO: 75 - protein, 24 aa, Homo sapiens
IYIWAPLAGTCGVLLLSLVITLYC

SEQ ID NO: 76 - DNA, 126 bp, Homo sapiens
aaacggggcagaaagaaactcctgtatatattcaaacaaccatttatgagaccagtacaaactactcaagaggaagatggctgtagctgccgatttccagaagaagaagaaggaggatgtgaactg

SEQ ID NO: 77 - protein, 42 aa, Homo sapiens
KRGRKKLLYIFKQPFMRPVQTTQEEDGCSCRFPEEEEGGCEL

SEQ ID NO: 78 - DNA, 336 bp, Homo sapiens
agagtgaagttcagcaggagcgcagacgcccccgcgtacaagcagggccagaaccagctctataacgagctcaatctaggacgaagagaggagtacgatgttttggacaagagacgtggccgggaccctgagatggggggaaagccgagaaggaagaaccctcaggaaggcctgtacaatgaactgcagaaagataagatggcggaggcctacagtgagattgggatgaaaggcgagcgccggaggggcaaggggcacgatggcctttaccagggtctcagtacagccaccaaggacacctacgacgcccttcacatgcaggccctgccccctcgc

SEQ ID NO: 79 - protein, 112 aa, Homo sapiens
RVKFSRSADAPAYKQGQNQLYNELNLGRREEYDVLDKRRGRDPEMGGKPRRKNPQEGLYNELQKDKMAEAYSEIGMKGERRRGKGHDGLYQGLSTATKDTYDALHMQALPPR

SEQ ID NO: 80 - DNA, 1503 bp, Artificial Sequence
  construct
atggccttaccagtgaccgccttgctcctgccgctggccttgctgctccacgccgccaggccgtctagacagtctgtgctgactcagccgccctcagtgtctggggccccagggcagagtgtcattatctcctgcactgggagcagctccaacatcggggcaggttctcatgtacactggtaccagcaggttccaggaacagcccccaaactcctcatctatgaaaacaccaatcggccctcaggggtccctgaccgattctctggctccaagtctggcacctcaggttccctggccatcactggactccagcctgaggatgaggctgattattattgtgcaacatgggatgacagtctgaatggtgtaatattcggcggagggaccaaggccaccgtcctaggcggatcctctaggtcaagttccagcggcggcggtggcagcggaggcggcggtgaggtgcagctggtggagtctgggggagccctggccaagcctggggggtccctgagactctcctgtgcagcctctggattcaccctcagtggctatgctatgcactgggtccgccaggctccaggcaaggggctggagtgggtggcagttatatcatatgatggaagcaataaatactacgcagactccgtgaagggccgattcaccgtctccagagacaattccaagaacacgctgtttctgcaaatgaacagcctgagacctgaggacacggctgtgtactattgtgctaaaggccttacctggggactcggtgacaatgatgctctcgatatctggggccccgggaccacggtcaccgtctcctcaagatccaccacgacgccagcgccgcgaccaccaacaccggcgcccaccatcgcgtcgcagcccctgtccctgcgcccagaggcgtgccggccagcggcggggggcgcagtgcacacgagggggctggacttcgcctgtgatatctacatctgggcgcccttggccgggacttgtggggtccttctcctgtcactggttatcaccctttactgcaaacggggcagaaagaaactcctgtatatattcaaacaaccatttatgagaccagtacaaactactcaagaggaagatggctgtagctgccgatttccagaagaagaagaaggaggatgtgaactgagagtgaagttcagcaggagcgcagacgcccccgcgtaccagcagggccagaaccagctctataacgagctcaatctaggacgaagagaggagtacgatgttttggacaagagacgtggccgggaccctgagatggggggaaagccgagaaggaagaaccctcaggaaggcctgtacaatgaactgcagaaagataagatggcggaggcctacagtgagattgggatgaaaggcgagcgccggaggggcaaggggcacgatggcctttaccagggtctcagtacagccaccaaggacacctacgacgcccttcacatgcaggccctgccccctcgctaa

SEQ ID NO: 81 - protein, 500 aa, Artificial Sequence
  construct
MALPVTALLLPLALLLHAARPSRQSVLTQPPSVSGAPGQSVIISCTGSSSNIGAGSHVHWYQQVPGTAPKLLIYENTNRPSGVPDRFSGSKSGTSGSLAITGLQPEDEADYYCATWDDSLNGVIFGGGTKATVLGGSSRSSSSGGGGSGGGGEVQLVESGGALAKPGGSLRLSCAASGFTLSGYAMHWVRQAPGKGLEWVAVISYDGSNKYYADSVKGRFTVSRDNSKNTLFLQMNSLRPEDTAVYYCAKGLTWGLGDNDALDIWGPGTTVTVSSRSTTTPAPRPPTPAPTIASQPLSLRPEACRPAAGGAVHTRGLDFACDIYIWAPLAGTCGVLLLSLVITLYCKRGRKKLLYIFKQPFMRPVQTTQEEDGCSCRFPEEEEGGCELRVKFSRSADAPAYQQGQNQLYNELNLGRREEYDVLDKRRGRDPEMGGKPRRKNPQEGLYNELQKDKMAEAYSEIGMKGERRRGKGHDGLYQGLSTATKDTYDALHMQALPPR

SEQ ID NO: 82 - DNA, 723 bp, Artificial Sequence
  scFv
caggtgcagctgcagcagagcggcgcggaactggcgcgcccgggcgcgagcgtgaaaatgagctgcaaagcgagcggctatacctttacccgctataccatgcattgggtgaaacagcgcccgggccagggcctggaatggattggctatattaacccgagccgcggctataccaactataaccagaaatttaaagataaagcgaccctgaccaccgataaaagcagcagcaccgcgtatatgcagctgagcagcctgaccagcgaagatagcgcggtgtattattgcgcgcgctattatgatgatcattattgcctggattattggggccagggcaccaccctgaccgtgagcagcggcggcggcggcagcggcggcggcggcagcggcggcggcggcagccagattgtgctgacccagagcccggcgattatgagcgcgagcccgggcgaaaaagtgaccatgacctgcagcgcgagcagcagcgtgagctatatgaactggtatcagcagaaaagcggcaccagcccgaaacgctggatttatgataccagcaaactggcgagcggcgtgccggcgcattttcgcggcagcggcagcggcaccagctatagcctgaccattagcggcatggaagcggaagatgcggcgacctattattgccagcagtggagcagcaacccgtttacctttggcagcggcaccaaactggaaattaaccgc

SEQ ID NO: 83 - protein, 241 aa, Artificial Sequence
  scFv
QVQLQQSGAELARPGASVKMSCKASGYTFTRYTMHWVKQRPGQGLEWIGYINPSRGYTNYNQKFKDKATLTTDKSSSTAYMQLSSLTSEDSAVYYCARYYDDHYCLDYWGQGTTLTVSSGGGGSGGGGSGGGGSQIVLTQSPAIMSASPGEKVTMTCSASSSVSYMNWYQQKSGTSPKRWIYDTSKLASGVPAHFRGSGSGTSYSLTISGMEAEDAATYYCQQWSSNPFTFGSGTKLEINR

SEQ ID NO: 84 - DNA, 357 bp, Mus musculus
caggtgcagctgcagcagagcggcgcggaactggcgcgcccgggcgcgagcgtgaaaatgagctgcaaagcgagcggctatacctttacccgctataccatgcattgggtgaaacagcgcccgggccagggcctggaatggattggctatattaacccgagccgcggctataccaactataaccagaaatttaaagataaagcgaccctgaccaccgataaaagcagcagcaccgcgtatatgcagctgagcagcctgaccagcgaagatagcgcggtgtattattgcgcgcgctattatgatgatcattattgcctggattattggggccagggcaccaccctgaccgtgagcagc

SEQ ID NO: 85 - protein, 119 aa, Mus musculus [sequence omitted]

SEQ ID NO: 86 - DNA, 321 bp, Mus musculus
cagattgtgctgacccagagcccggcgattatgagcgcgagcccgggcgaaaaagtgaccatgacctgcagcgcgagcagcagcgtgagctatatgaactggtatcagcagaaaagcggcaccagcccgaaacgctggatttatgataccagcaaactggcgagcggcgtgccggcgcattttcgcggcagcggcagcggcaccagctatagcctgaccattagcggcatggaagcggaagatgcggcgacctattattgccagcagtggagcagcaacccgtttacctttggcagcggcaccaaactggaaattaaccgc

SEQ ID NO: 87 - protein, 107 aa, Mus musculus
QIVLTQSPAIMSASPGEKVTMTCSASSSVSYMNWYQQKSGTSPKRWIYDTSKLASGVPAHFRGSGSGTSYSLTISGMEAEDAATYYCQQWSSNPFTFGSGTKLEINR

SEQ ID NO: 88 - DNA, 723 bp, Artificial Sequence
  humanized scFv
caggtgcagctggtgcagagcggcggcggcgtggtgcagccgggccgcagcctgcgcctgagctgcaaagcgagcggctatacctttacccgctataccatgcattgggtgcgccaggcgccgggcaaaggcctggaatggattggctatattaacccgagccgcggctataccaactataaccagaaagtgaaagatcgctttaccattagcaccgataaaagcaaaagcaccgcgtttctgcagatggatagcctgcgcccggaagataccggcgtgtatttttgcgcgcgctattatgatgatcattattgcctggattattggggccagggcaccaccctgaccgtgagcagcggcggcggcggcagcggcggcggcggcagcggcggcggcggcagcgatattcagatgacccagagcccgagcagcctgagcgcgagcgtgggcgatcgcgtgaccattacctgcagcgcgagcagcagcgtgagctatatgaactggtatcagcagaccccgggcaaagcgccgaaacgctggatttatgataccagcaaactggcgagcggcgtgccgagccgctttagcggcagcggcagcggcaccgattatacctttaccattagcagcctgcagccggaagatattgcgacctattattgccagcagtggagcagcaacccgtttacctttggccagggcaccaaactgcagattacccgc

SEQ ID NO: 89 - protein, 241 aa, Artificial Sequence
  humanized scFv
QVQLVQSGGGVVQPGRSLRLSCKASGYTFTRYTMHWVRQAPGKGLEWIGYINPSRGYTNYNQKVKDRFTISTDKSKSTAFLQMDSLRPEDTGVYFCARYYDDHYCLDYWGQGTTLTVSSGGGGSGGGGSGGGGSDIQMTQSPSSLSASVGDRVTITCSASSSVSYMNWYQQTPGKAPKRWIYDTSKLASGVPSRFSGSGSGTDYTFTISSLQPEDIATYYCQQWSSNPFTFGQGTKLQITR

SEQ ID NO: 90 - DNA, 357 bp, Homo sapiens
caggtgcagctggtgcagagcggcggcggcgtggtgcagccgggccgcagcctgcgcctgagctgcaaagcgagcggctatacctttacccgctataccatgcattgggtgcgccaggcgccgggcaaaggcctggaatggattggctatattaacccgagccgcggctataccaactataaccagaaagtgaaagatcgctttaccattagcaccgataaaagcaaaagcaccgcgtttctgcagatggatagcctgcgcccggaagataccggcgtgtatttttgcgcgcgctattatgatgatcattattgcctggattattggggccagggcaccaccctgaccgtgagcagc

SEQ ID NO: 91 - protein, 119 aa, Homo sapiens
QVQLVQSGGGVVQPGRSLRLSCKASGYTFTRYTMHWVRQAPGKGLEWIGYINPSRGYTNYNQKVKDRFTISTDKSKSTAFLQMDSLRPEDTGVYFCARYYDDHYCLDYWGQGTTLTVSS

SEQ ID NO: 92 - DNA, 321 bp, Homo sapiens
gatattcagatgacccagagcccgagcagcctgagcgcgagcgtgggcgatcgcgtgaccattacctgcagcgcgagcagcagcgtgagctatatgaactggtatcagcagaccccgggcaaagcgccgaaacgctggatttatgataccagcaaactggcgagcggcgtgccgagccgctttagcggcagcggcagcggcaccgattatacctttaccattagcagcctgcagccggaagatattgcgacctattattgccagcagtggagcagcaacccgtttacctttggccagggcaccaaactgcagattacccgc

SEQ ID NO: 93 - protein, 107 aa, Homo sapiens
DIQMTQSPSSLSASVGDRVTITCSASSSVSYMNWYQQTPGKAPKRWIYDTSKLASGVPSRFSGSGSGTDYTFTISSLQPEDIATYYCQQWSSNPFTFGQGTKLQITR

SEQ ID NO: 94 - DNA, 45 bp, Artificial Sequence
  mutant
gagcccaaatctgctgacaaaactcacacatgcccaccgtgccca

SEQ ID NO: 95 - protein, 15 aa, Artificial Sequence
  mutated IgG1 hinge amino acid sequence
EPKSADKTHTCPPCP

SEQ ID NO: 96 - DNA, 651 bp, Artificial Sequence
  mutated IgG4 Fc (N297A) nucleic acid sequence
gcacctgagttcctggggggaccatcagtcttcctgttccccccaaaacccaaggacactctcatgatctcccggacccctgaggtcacgtgcgtggtggtggacgtgagccaggaagaccccgaggtccagttcaactggtacgtggatggcgtggaggtgcataatgccaagacaaagccgcgggaggagcagttcgctagcacgtaccgtgtggtcagcgtcctcaccgtcctgcaccaggactggctgaacggcaaggagtacaagtgcaaggtctccaacaaaggcctcccgtcctccatcgagaaaaccatctccaaagccaaagggcagccccgagagccacaggtgtacaccctgcccccatcccaggaggagatgaccaagaaccaggtcagcctgacctgcctggtcaaaggcttctaccccagcgacatcgccgtggagtgggagagcaatgggcagccggagaacaactacaagaccacgcctcccgtgctggactccgacggctccttcttcctctacagcaggctaaccgtggacaagagcaggtggcaggaggggaatgtcttctcatgctccgtgatgcatgaggctctgcacaaccactacacacagaagagcctctccctgtctctgggtaaa

SEQ ID NO: 97 - protein, 217 aa, Artificial Sequence
  mutated IgG4 Fc (N297A) amino acid sequence
APEFLGGPSVFLFPPKPKDTLMISRTPEVTCVVVDVSQEDPEVQFNWYVDGVEVHNAKTKPREEQFASTYRVVSVLTVLHQDWLNGKEYKCKVSNKGLPSSIEKTISKAKGQPREPQVYTLPPSQEEMTKNQVSLTCLVKGFYPSDIAVEWESNGQPENNYKTTPPVLDSDGSFFLYSRLTVDKSRWQEGNVFSCSVMHEALHNHYTQKSLSLSLGK

SEQ ID NO: 98 - DNA, 696 bp, Artificial Sequence
  mutated IgG1 Hinge-IgG4 Fc nucleic acid sequence
gagcccaaatctgctgacaaaactcacacatgcccaccgtgcccagcacctgagttcctggggggaccatcagtcttcctgttccccccaaaacccaaggacactctcatgatctcccggacccctgaggtcacgtgcgtggtggtggacgtgagccaggaagaccccgaggtccagttcaactggtacgtggatggcgtggaggtgcataatgccaagacaaagccgcgggaggagcagttcgctagcacgtaccgtgtggtcagcgtcctcaccgtcctgcaccaggactggctgaacggcaaggagtacaagtgcaaggtctccaacaaaggcctcccgtcctccatcgagaaaaccatctccaaagccaaagggcagccccgagagccacaggtgtacaccctgcccccatcccaggaggagatgaccaagaaccaggtcagcctgacctgcctggtcaaaggcttctaccccagcgacatcgccgtggagtgggagagcaatgggcagccggagaacaactacaagaccacgcctcccgtgctggactccgacggctccttcttcctctacagcaggctaaccgtggacaagagcaggtggcaggaggggaatgtcttctcatgctccgtgatgcatgaggctctgcacaaccactacacacagaagagcctctccctgtctctgggtaaa

SEQ ID NO: 99 - protein, 232 aa, Artificial Sequence
  mutated IgG1 Hinge-IgG4 Fc amino acid sequence
EPKSADKTHTCPPCPAPEFLGGPSVFLFPPKPKDTLMISRTPEVTCVVVDVSQEDPEVQFNWYVDGVEVHNAKTKPREEQFASTYRVVSVLTVLHQDWLNGKEYKCKVSNKGLPSSIEKTISKAKGQPREPQVYTLPPSQEEMTKNQVSLTCLVKGFYPSDIAVEWESNGQPENNYKTTPPVLDSDGSFFLYSRLTVDKSRWQEGNVFSCSVMHEALHNHYTQKSLSLSLGK

SEQ ID NO: 100 - DNA, 1547 bp, Artificial Sequence
  scFv1 MCS-G4S-hOKT3 scFv-IgG1 hinge - IgG4 Fc expression cassette nucleic acid sequence
actagtgccaccatggagtttgggctgagctgggtcttcctggtggctatcttgaagggtgtccagtgtgaattcaagctttctagaagcgctgctagcggtggaggtggatcccaggtccagctggtgcagtcaggggggggagtcgtgcagcccggtcggtctctgcgtctgtcttgtaaggcatccggttatacttttaccaggtacacaatgcactgggtgcggcaggctcctggcaagggcctggagtggatcggctatatcaacccatccaggggctacaccaactataatcagaaggtgaaggaccggttcaccatctctacagataagagcaagtctacagcctttctgcagatggactccctgagacctgaggataccggcgtgtacttctgcgctcgctactatgacgatcattactgtctggactattggggccagggcaccacactgacagtgtccagcggaggaggaggctccggaggaggaggcagcggcggcggcggctctgacatccagatgacccagagcccatcttccctgtccgccagcgtgggcgatagagtgaccatcacatgctccgcctcctcctccgtgtcctacatgaactggtatcagcagacacccggcaaggcccctaagagatggatctacgatacctccaagctggcctccggagtgccctctcgcttctctggctccggcagcggcacagactatacctttacaatcagctctctgcagcctgaggatatcgctacctactattgtcagcagtggtccagcaatccattcacctttggccagggcacaaagctgcagatcaccaggctcgagccaaagagcgccgacaagacccacacatgccccccttgtccagctcccgagtttctgggcggcccatccgtgttcctgtttccacccaagcccaaggatacactgatgatcagccggaccccagaggtgacatgcgtggtggtggacgtgtctcaggaggaccccgaggtgcagttcaactggtacgtggacggcgtggaggtgcacaatgccaagaccaagcccagggaggagcagtttgcttctacataccgggtggtgtccgtgctgaccgtgctgcatcaggattggctgaacggcaaggagtataagtgcaaggtgtccaataagggcctgccttcttccatcgagaagacaatcagcaaggctaagggacagcctcgcgagccacaggtgtacaccctgcctccatctcaggaggagatgacaaagaaccaggtgtccctgacctgtctggtgaagggcttctatccctccgacatcgctgtggagtgggagagcaatggccagcctgagaacaattacaagaccacaccccctgtgctggacagcgatggctctttctttctgtatagcagactgaccgtggataagtctcgctggcaggagggcaacgtgttctcctgttccgtgatgcacgaggcactgcacaaccactacactcagaaatcactgtcactgtccctgggcaagtaggcggccgc

SEQ ID NO: 101 - protein, 496 aa, Artificial Sequence
  scFv1 MCS-G4S-hOKT3 scFv-IgG1 hinge - IgG4 Fc expression cassette amino acid sequence
MEFGLSWVFLVAILKGVQCMCSQVQLVQSGGGVVQPGRSLRLSCKASGYTFTRYTMHWVRQAPGKGLEWIGYINPSRGYTNYNQKVKDRFTISTDKSKSTAFLQMDSLRPEDTGVYFCARYYDDHYCLDYWGQGTTLTVSSGGGGSGGGGSGGGGSDIQMTQSPSSLSASVGDRVTITCSASSSVSYMNWYQQTPGKAPKRWIYDTSKLASGVPSRFSGSGSGTDYTFTISSLQPEDIATYYCQQWSSNPFTFGQGTKLQITRLEPKSADKTHTCPPCPAPEFLGGPSVFLFPPKPKDTLMISRTPEVTCVVVDVSQEDPEVQFNWYVDGVEVHNAKTKPREEQFASTYRVVSVLTVLHQDWLNGKEYKCKVSNKGLPSSIEKTISKAKGQPREPQVYTLPPSQEEMTKNQVSLTCLVKGFYPSDIAVEWESNGQPENNYKTTPPVLDSDGSFFLYSRLTVDKSRWQEGNVFSCSVMHEALHNHYTQKSLSLSLGK

SEQ ID NO: 102 - DNA, 1547 bp, Artificial Sequence
  scFv1 MCS-G4S-mOKT3 scFv-IgG1 hinge - IgG4 Fc expression cassette nucleic acid sequence
actagtgccaccatggagtttgggctgagctgggtcttcctggtggctatcttgaagggtgtccagtgtgaattcaagctttctagaagcgctgctagcggtggaggtggatcccaggtccagctgcagcagagcggtgccgaactggcccgtcccggagcaagcgtgaaaatgtcctgtaaagcaagtggctataccttcaccaggtacacaatgcactgggtgaagcagaggccaggacagggcctggagtggatcggctatatcaacccctctaggggctacacaaactataatcagaagttcaaggacaaggccaccctgaccaccgataagtccagctctacagcttacatgcagctgtccagcctgaccagcgaggactctgccgtgtactattgcgctagatactatgacgatcattactgtctggattattggggccagggcaccacactgacagtgtcttccggaggaggaggcagcggaggaggaggctctggcggcggcggctcccagatcgtgctgacccagtccccagctatcatgtccgcctcccctggagagaaggtgaccatgacatgcagcgccagctcttccgtgtcttacatgaattggtatcagcagaagtccggcacaagccctaagagatggatctacgacacctctaagctggcctccggagtgccagctcactttcgcggctccggcagcggcacctcttattccctgacaatcagcggcatggaggctgaggatgccgctacctactattgtcagcagtggtcatcaaatcctttcaccttcggttcagggacaaaactggagatcaataggctcgagccaaagagcgccgacaagacccacacatgccccccttgtccagctcccgagtttctgggcggcccatccgtgttcctgtttccacccaagcccaaggatacactgatgatcagccggaccccagaggtgacatgcgtggtggtggacgtgtctcaggaggaccccgaggtgcagttcaactggtacgtggacggcgtggaggtgcacaatgccaagaccaagcccagggaggagcagtttgcttctacataccgggtggtgtccgtgctgaccgtgctgcatcaggattggctgaacggcaaggagtataagtgcaaggtgtccaataagggcctgccttcttccatcgagaagacaatcagcaaggctaagggacagcctcgcgagccacaggtgtacaccctgcctccatctcaggaggagatgacaaagaaccaggtgtccctgacctgtctggtgaagggcttctatccctccgacatcgctgtggagtgggagagcaatggccagcctgagaacaattacaagaccacaccccctgtgctggacagcgatggctctttctttctgtatagcagactgaccgtggataagtctcgctggcaggagggcaacgtgttctcctgttccgtgatgcacgaggcactgcacaaccactacactcagaaatcactgtcactgtccctgggcaagtaggcggccgc

SEQ ID NO: 103 - protein, 496 aa, Artificial Sequence
  scFv1 MCS-G4S-mOKT3 scFv-IgG1 hinge - IgG4 Fc expression cassette amino acid sequence
MEFGLSWVFLVAILKGVQCMCSQVQLQQSGAELARPGASVKMSCKASGYTFTRYTMHWVKQRPGQGLEWIGYINPSRGYTNYNQKFKDKATLTTDKSSSTAYMQLSSLTSEDSAVYYCARYYDDHYCLDYWGQGTTLTVSSGGGGSGGGGSGGGGSQIVLTQSPAIMSASPGEKVTMTCSASSSVSYMNWYQQKSGTSPKRWIYDTSKLASGVPAHFRGSGSGTSYSLTISGMEAEDAATYYCQQWSSNPFTFGSGTKLEINRLEPKSADKTHTCPPCPAPEFLGGPSVFLFPPKPKDTLMISRTPEVTCVVVDVSQEDPEVQFNWYVDGVEVHNAKTKPREEQFASTYRVVSVLTVLHQDWLNGKEYKCKVSNKGLPSSIEKTISKAKGQPREPQVYTLPPSQEEMTKNQVSLTCLVKGFYPSDIAVEWESNGQPENNYKTTPPVLDSDGSFFLYSRLTVDKSRWQEGNVFSCSVMHEALHNHYTQKSLSLSLGK

SEQ ID NO: 104 - DNA, 2265 bp, Artificial Sequence
  anti-PSMA & hOKT3 bispecific Ab nucleic acid sequence (gy1-2)
atggagtttgggctgagctgggtcttcctggtggctatcttgaagggtgtccagtgtgaattccagtctgtgctgactcagccgccctcagtgtctggggccccagggcagagtgtcattatctcctgcactgggagcagctccaacatcggggcaggttctcatgtacactggtaccagcaggttccaggaacagcccccaaactcctcatctatgaaaacaccaatcggccctcaggggtccctgaccgattctctggctccaagtctggcacctcaggttccctggccatcactggactccagcctgaggatgaggctgattattattgtgcaacatgggatgacagtctgaatggtgtaatattcggcggagggaccaaggccaccgtcctaggcggatcctctaggtcaagttccagcggcggcggtggcagcggaggcggcggtgaggtgcagctggtggagtctgggggagccctggccaagcctggggggtccctgagactctcctgtgcagcctctggattcaccctcagtggctatgctatgcactgggtccgccaggctccaggcaaggggctggagtgggtggcagttatatcatatgatggaagcaataaatactacgcagactccgtgaagggccgattcaccgtctccagagacaattccaagaacacgctgtttctgcaaatgaacagcctgagacctgaggacacggctgtgtactattgtgctaaaggccttacctggggactcggtgacaatgatgctctcgatatctggggccccgggaccacggtcaccgtctcctcagctagcggtggaggtggatcccaggtccagctggtgcagtcaggggggggagtcgtgcagcccggtcggtctctgcgtctgtcttgtaaggcatccggttatacttttaccaggtacacaatgcactgggtgcggcaggctcctggcaagggcctggagtggatcggctatatcaacccatccaggggctacaccaactataatcagaaggtgaaggaccggttcaccatctctacagataagagcaagtctacagcctttctgcagatggactccctgagacctgaggataccggcgtgtacttctgcgctcgctactatgacgatcattactgtctggactattggggccagggcaccacactgacagtgtccagcggaggaggaggctccggaggaggaggcagcggcggcggcggctctgacatccagatgacccagagcccatcttccctgtccgccagcgtgggcgatagagtgaccatcacatgctccgcctcctcctccgtgtcctacatgaactggtatcagcagacacccggcaaggcccctaagagatggatctacgatacctccaagctggcctccggagtgccctctcgcttctctggctccggcagcggcacagactatacctttacaatcagctctctgcagcctgaggatatcgctacctactattgtcagcagtggtccagcaatccattcacctttggccagggcacaaagctgcagatcaccaggctcgagccaaagagcgccgacaagacccacacatgccccccttgtccagctcccgagtttctgggcggcccatccgtgttcctgtttccacccaagcccaaggatacactgatgatcagccggaccccagaggtgacatgcgtggtggtggacgtgtctcaggaggaccccgaggtgcagttcaactggtacgtggacggcgtggaggtgcacaatgccaagaccaagcccagggaggagcagtttgcttctacataccgggtggtgtccgtgctgaccgtgctgcatcaggattggctgaacggcaaggagtataagtgcaaggtgtccaataagggcctgccttcttccatcgagaagacaatcagcaaggctaagggacagcctcgcgagccacaggtgtacaccctgcctccatctcaggaggagatgacaaagaaccaggtgtccctgacctgtctggtgaagggcttctatccctccgacatcgctgtggagtgggagagcaatggccagcctgagaacaattacaagaccacaccccctgtgctggacagcgatggctctttctttctgtatagcagactgaccgtggataagtctcgctggcaggagggcaacgtgttctcctgttccgtgatgcacgaggcactgcacaaccactacactcagaaatcactgtcactgtccctgggcaagtag

SEQ ID NO: 105 - protein, 754 aa, Artificial Sequence
  anti-PSMA & hOKT3 bispecific Ab amino acid sequence (gy1-2)
MEFGLSWVFLVAILKGVQCEFQSVLTQPPSVSGAPGQSVIISCTGSSSNIGAGSHVHWYQQVPGTAPKLLIYENTNRPSGVPDRFSGSKSGTSGSLAITGLQPEDEADYYCATWDDSLNGVIFGGGTKATVLGGSSRSSSSGGGGSGGGGEVQLVESGGALAKPGGSLRLSCAASGFTLSGYAMHWVRQAPGKGLEWVAVISYDGSNKYYADSVKGRFTVSRDNSKNTLFLQMNSLRPEDTAVYYCAKGLTWGLGDNDALDIWGPGTTVTVSSASGGGGSQVQLVQSGGGVVQPGRSLRLSCKASGYTFTRYTMHWVRQAPGKGLEWIGYINPSRGYTNYNQKVKDRFTISTDKSKSTAFLQMDSLRPEDTGVYFCARYYDDHYCLDYWGQGTTLTVSSGGGGSGGGGSGGGGSDIQMTQSPSSLSASVGDRVTITCSASSSVSYMNWYQQTPGKAPKRWIYDTSKLASGVPSRFSGSGSGTDYTFTISSLQPEDIATYYCQQWSSNPFTFGQGTKLQITRLEPKSADKTHTCPPCPAPEFLGGPSVFLFPPKPKDTLMISRTPEVTCVVVDVSQEDPEVQFNWYVDGVEVHNAKTKPREEQFASTYRVVSVLTVLHQDWLNGKEYKCKVSNKGLPSSIEKTISKAKGQPREPQVYTLPPSQEEMTKNQVSLTCLVKGFYPSDIAVEWESNGQPENNYKTTPPVLDSDGSFFLYSRLTVDKSRWQEGNVFSCSVMHEALHNHYTQKSLSLSLGK

SEQ ID NO: 106 - protein, 735 aa, Artificial Sequence
  anti-PSMA & hOKT3 bispecific Ab amino acid sequence (gy1-2) without signal peptide
EFQSVLTQPPSVSGAPGQSVIISCTGSSSNIGAGSHVHWYQQVPGTAPKLLIYENTNRPSGVPDRFSGSKSGTSGSLAITGLQPEDEADYYCATWDDSLNGVIFGGGTKATVLGGSSRSSSSGGGGSGGGGEVQLVESGGALAKPGGSLRLSCAASGFTLSGYAMHWVRQAPGKGLEWVAVISYDGSNKYYADSVKGRFTVSRDNSKNTLFLQMNSLRPEDTAVYYCAKGLTWGLGDNDALDIWGPGTTVTVSSASGGGGSQVQLVQSGGGVVQPGRSLRLSCKASGYTFTRYTMHWVRQAPGKGLEWIGYINPSRGYTNYNQKVKDRFTISTDKSKSTAFLQMDSLRPEDTGVYFCARYYDDHYCLDYWGQGTTLTVSSGGGGSGGGGSGGGGSDIQMTQSPSSLSASVGDRVTITCSASSSVSYMNWYQQTPGKAPKRWIYDTSKLASGVPSRFSGSGSGTDYTFTISSLQPEDIATYYCQQWSSNPFTFGQGTKLQITRLEPKSADKTHTCPPCPAPEFLGGPSVFLFPPKPKDTLMISRTPEVTCVVVDVSQEDPEVQFNWYVDGVEVHNAKTKPREEQFASTYRVVSVLTVLHQDWLNGKEYKCKVSNKGLPSSIEKTISKAKGQPREPQVYTLPPSQEEMTKNQVSLTCLVKGFYPSDIAVEWESNGQPENNYKTTPPVLDSDGSFFLYSRLTVDKSRWQEGNVFSCSVMHEALHNHYTQKSLSLSLGK

SEQ ID NO: 107 - DNA, 2265 bp, Artificial Sequence
  anti-PSMA & mOKT3 bispecific Ab nucleic acid sequence (gy1-2)
atggagtttgggctgagctgggtcttcctggtggctatcttgaagggtgtccagtgtgaattccagtctgtgctgactcagccgccctcagtgtctggggccccagggcagagtgtcattatctcctgcactgggagcagctccaacatcggggcaggttctcatgtacactggtaccagcaggttccaggaacagcccccaaactcctcatctatgaaaacaccaatcggccctcaggggtccctgaccgattctctggctccaagtctggcacctcaggttccctggccatcactggactccagcctgaggatgaggctgattattattgtgcaacatgggatgacagtctgaatggtgtaatattcggcggagggaccaaggccaccgtcctaggcggatcctctaggtcaagttccagcggcggcggtggcagcggaggcggcggtgaggtgcagctggtggagtctgggggagccctggccaagcctggggggtccctgagactctcctgtgcagcctctggattcaccctcagtggctatgctatgcactgggtccgccaggctccaggcaaggggctggagtgggtggcagttatatcatatgatggaagcaataaatactacgcagactccgtgaagggccgattcaccgtctccagagacaattccaagaacacgctgtttctgcaaatgaacagcctgagacctgaggacacggctgtgtactattgtgctaaaggccttacctggggactcggtgacaatgatgctctcgatatctggggccccgggaccacggtcaccgtctcctcagctagcggtggaggtggatcccaggtccagctgcagcagagcggtgccgaactggcccgtcccggagcaagcgtgaaaatgtcctgtaaagcaagtggctataccttcaccaggtacacaatgcactgggtgaagcagaggccaggacagggcctggagtggatcggctatatcaacccctctaggggctacacaaactataatcagaagttcaaggacaaggccaccctgaccaccgataagtccagctctacagcttacatgcagctgtccagcctgaccagcgaggactctgccgtgtactattgcgctagatactatgacgatcattactgtctggattattggggccagggcaccacactgacagtgtcttccggaggaggaggcagcggaggaggaggctctggcggcggcggctcccagatcgtgctgacccagtccccagctatcatgtccgcctcccctggagagaaggtgaccatgacatgcagcgccagctcttccgtgtcttacatgaattggtatcagcagaagtccggcacaagccctaagagatggatctacgacacctctaagctggcctccggagtgccagctcactttcgcggctccggcagcggcacctcttattccctgacaatcagcggcatggaggctgaggatgccgctacctactattgtcagcagtggtcatcaaatcctttcaccttcggttcagggacaaaactggagatcaataggctcgagccaaagagcgccgacaagacccacacatgccccccttgtccagctcccgagtttctgggcggcccatccgtgttcctgtttccacccaagcccaaggatacactgatgatcagccggaccccagaggtgacatgcgtggtggtggacgtgtctcaggaggaccccgaggtgcagttcaactggtacgtggacggcgtggaggtgcacaatgccaagaccaagcccagggaggagcagtttgcttctacataccgggtggtgtccgtgctgaccgtgctgcatcaggattggctgaacggcaaggagtataagtgcaaggtgtccaataagggcctgccttcttccatcgagaagacaatcagcaaggctaagggacagcctcgcgagccacaggtgtacaccctgcctccatctcaggaggagatgacaaagaaccaggtgtccctgacctgtctggtgaagggcttctatccctccgacatcgctgtggagtgggagagcaatggccagcctgagaacaattacaagaccacaccccctgtgctggacagcgatggctctttctttctgtatagcagactgaccgtggataagtctcgctggcaggagggcaacgtgttctcctgttccgtgatgcacgaggcactgcacaaccactacactcagaaatcactgtcactgtccctgggcaagtag

SEQ ID NO: 108 - protein, 754 aa, Artificial Sequence
  anti-PSMA & mOKT3 bispecific Ab amino acid sequence (gy1-2)
MEFGLSWVFLVAILKGVQCEFQSVLTQPPSVSGAPGQSVIISCTGSSSNIGAGSHVHWYQQVPGTAPKLLIYENTNRPSGVPDRFSGSKSGTSGSLAITGLQPEDEADYYCATWDDSLNGVIFGGGTKATVLGGSSRSSSSGGGGSGGGGEVQLVESGGALAKPGGSLRLSCAASGFTLSGYAMHWVRQAPGKGLEWVAVISYDGSNKYYADSVKGRFTVSRDNSKNTLFLQMNSLRPEDTAVYYCAKGLTWGLGDNDALDIWGPGTTVTVSSASGGGGSQVQLQQSGAELARPGASVKMSCKASGYTFTRYTMHWVKQRPGQGLEWIGYINPSRGYTNYNQKFKDKATLTTDKSSSTAYMQLSSLTSEDSAVYYCARYYDDHYCLDYWGQGTTLTVSSGGGGSGGGGSGGGGSQIVLTQSPAIMSASPGEKVTMTCSASSSVSYMNWYQQKSGTSPKRWIYDTSKLASGVPAHFRGSGSGTSYSLTISGMEAEDAATYYCQQWSSNPFTFGSGTKLEINRLEPKSADKTHTCPPCPAPEFLGGPSVFLFPPKPKDTLMISRTPEVTCVVVDVSQEDPEVQFNWYVDGVEVHNAKTKPREEQFASTYRVVSVLTVLHQDWLNGKEYKCKVSNKGLPSSIEKTISKAKGQPREPQVYTLPPSQEEMTKNQVSLTCLVKGFYPSDIAVEWESNGQPENNYKTTPPVLDSDGSFFLYSRLTVDKSRWQEGNVFSCSVMHEALHNHYTQKSLSLSLGK

SEQ ID NO: 109 - protein, 735 aa, Artificial Sequence
  anti-PSMA & mOKT3 bispecific Ab amino acid sequence (gy1-2)
EFQSVLTQPPSVSGAPGQSVIISCTGSSSNIGAGSHVHWYQQVPGTAPKLLIYENTNRPSGVPDRFSGSKSGTSGSLAITGLQPEDEADYYCATWDDSLNGVIFGGGTKATVLGGSSRSSSSGGGGSGGGGEVQLVESGGALAKPGGSLRLSCAASGFTLSGYAMHWVRQAPGKGLEWVAVISYDGSNKYYADSVKGRFTVSRDNSKNTLFLQMNSLRPEDTAVYYCAKGLTWGLGDNDALDIWGPGTTVTVSSASGGGGSQVQLQQSGAELARPGASVKMSCKASGYTFTRYTMHWVKQRPGQGLEWIGYINPSRGYTNYNQKFKDKATLTTDKSSSTAYMQLSSLTSEDSAVYYCARYYDDHYCLDYWGQGTTLTVSSGGGGSGGGGSGGGGSQIVLTQSPAIMSASPGEKVTMTCSASSSVSYMNWYQQKSGTSPKRWIYDTSKLASGVPAHFRGSGSGTSYSLTISGMEAEDAATYYCQQWSSNPFTFGSGTKLEINRLEPKSADKTHTCPPCPAPEFLGGPSVFLFPPKPKDTLMISRTPEVTCVVVDVSQEDPEVQFNWYVDGVEVHNAKTKPREEQFASTYRVVSVLTVLHQDWLNGKEYKCKVSNKGLPSSIEKTISKAKGQPREPQVYTLPPSQEEMTKNQVSLTCLVKGFYPSDIAVEWESNGQPENNYKTTPPVLDSDGSFFLYSRLTVDKSRWQEGNVFSCSVMHEALHNHYTQKSLSLSLGK

SEQ ID NO: 110 - DNA, 1184 bp, Homo sapiens
cgtgaggctccggtgcccgtcagtgggcagagcgcacatcgcccacagtccccgagaagttggggggaggggtcggcaattgaaccggtgcctagagaaggtggcgcggggtaaactgggaaagtgatgtcgtgtactggctccgcctttttcccgagggtgggggagaaccgtatataagtgcagtagtcgccgtgaacgttctttttcgcaacgggtttgccgccagaacacaggtaagtgccgtgtgtggttcccgcgggcctggcctctttacgggttatggcccttgcgtgccttgaattacttccacctggctgcagtacgtgattcttgatcccgagcttcgggttggaagtgggtgggagagttcgaggccttgcgcttaaggagccccttcgcctcgtgcttgagttgaggcctggcctgggcgctggggccgccgcgtgcgaatctggtggcaccttcgcgcctgtctcgctgctttcgataagtctctagccatttaaaatttttgatgacctgctgcgacgctttttttctggcaagatagtcttgtaaatgcgggccaagatctgcacactggtatttcggtttttggggccgcgggcggcgacggggcccgtgcgtcccagcgcacatgttcggcgaggcggggcctgcgagcgcggccaccgagaatcggacgggggtagtctcaagctggccggcctgctctggtgcctggcctcgcgccgccgtgtatcgccccgccctgggcggcaaggctggcccggtcggcaccagttgcgtgagcggaaagatggccgcttcccggccctgctgcagggagctcaaaatggaggacgcggcgctcgggagagcgggcgggtgagtcacccacacaaaggaaaagggcctttccgtcctcagccgtcgcttcatgtgactccacggagtaccgggcgccgtccaggcacctcgattagttctcgagcttttggagtacgtcgtctttaggttggggggaggggttttatgcgatggagtttccccacactgagtgggtggagactgaagttaggccagcttggcacttgatgtaattctccttggaatttgccctttttgagtttggatcttggttcattctcaagcctcagacagtggttcaaagtttttttcttccatttcaggtgtcgtga

SEQ ID NO: 111 - DNA, 21 bp, Artificial Sequence
  primer
gactacaaggacgacgatgac

SEQ ID NO: 112 - DNA, 25 bp, Artificial Sequence
  primer
agtagaatcaagacctagtagaggg

SEQ ID NO: 113 - DNA, 19 bp, Artificial Sequence
  primer
ctattgccagcattgctgc

SEQ ID NO: 114 - DNA, 20 bp, Artificial Sequence
  primer
atagggacctagacttcagg

SEQ ID NO: 115 - DNA, 20 bp, Artificial Sequence
  primer
ccttctactcctcctacacc

SEQ ID NO: 116 - DNA, 19 bp, Artificial Sequence
  primer
ggagggcgtgaatgtaagc